European Patent Specification EP 3 548 082 B1, published May 15, 2024. Title: A Method of Averting Opioid Addiction. Applicant: Regeneron Pharmaceuticals, Inc. Application TBA (Filed Herewith). The sequence listing filed with the application follows.

SEQUENCE LISTING (18 sequences)

SEQ ID NO: 1 - DNA, 357 bp, Artificial Sequence
  synthetic
caggtgcagctggtgcagtctggggctgaggtgaagaagcctggggcctcagtgaaggtctcctgcaaggtttccggattcaccctcactgaattatccattcactgggtgcgacaggctcctggaaaagggcttgagtggatgggaggttttgatcctgaagatggtgaaacaatctacgcacagaagttccagggcagagtcaccatgaccgaggacacatctacagacacagcctacatggagctgaccagcctgagatcggaagacacggccgtgtattactgttcaacgatttttggagtggttaccaactttgacaactggggccagggaaccctggtcaccgtctcctca

SEQ ID NO: 2 - protein, 119 aa, Artificial Sequence [sequence omitted]

SEQ ID NO: 3 - DNA, 24 bp, Artificial Sequence
  synthetic
ggattcaccctcactgaattatcc

SEQ ID NO: 4 - protein, 8 aa, Artificial Sequence
  synthetic
GFTLTELS

SEQ ID NO: 5 - DNA, 24 bp, Artificial Sequence
  synthetic
tttgatcctgaagatggtgaaaca

SEQ ID NO: 6 - protein, 8 aa, Artificial Sequence
  synthetic
FDPEDGET

SEQ ID NO: 7 - DNA, 36 bp, Artificial Sequence
  synthetic
tcaacgatttttggagtggttaccaactttgacaac

SEQ ID NO: 8 - protein, 12 aa, Artificial Sequence
  synthetic
STIFGVVTNFDN

SEQ ID NO: 9 - DNA, 324 bp, Artificial Sequence
  synthetic
gacatccagatgacccagtctccatcctccctgtctgcatctgcaggagacagagtcaccatcacttgccgggcaagtcaggccattagaaatgatttaggctggtatcagcagaaaccagggaaagcccctaagcgcctgatctatgctgcattcaatttgcaaagtggggtcccatcaagattcagcggcagtggatctgggacagaattcactctcacaatcagtagcctgcagcctgaagatcttgcaagttattactgtcaacagtataatagatacccgtggacgttcggccaagggaccaaggtggaaatcaaacga

SEQ ID NO: 10 - protein, 108 aa, Artificial Sequence
  synthetic
DIQMTQSPSSLSASAGDRVTITCRASQAIRNDLGWYQQKPGKAPKRLIYAAFNLQSGVPSRFSGSGSGTEFTLTISSLQPEDLASYYCQQYNRYPWTFGQGTKVEIKR

SEQ ID NO: 11 - DNA, 18 bp, Artificial Sequence
  synthetic
caggccattagaaatgat

SEQ ID NO: 12 - protein, 6 aa, Artificial Sequence
  synthetic
QAIRND

SEQ ID NO: 13 - DNA, 9 bp, Artificial Sequence
  synthetic
gctgcattc

SEQ ID NO: 14 - protein, 3 aa, Artificial Sequence
  synthetic
AAF

SEQ ID NO: 15 - DNA, 27 bp, Artificial Sequence
  synthetic
caacagtataatagatacccgtggacg

SEQ ID NO: 16 - protein, 9 aa, Artificial Sequence
  synthetic
QQYNRYPWT

SEQ ID NO: 17 - DNA, 847 bp, Artificial Sequence
  synthetic
agcgtccggacccaataacagttttaccaagggagcagctttctatcctggccacactgaggtgcatagcgtaatgtccatgttgttctacactctgatcacagcttttctgatcggcatacaggcggaaccacactcagagagcaatgtccctgcaggacacaccatcccccaagcccactggactaaacttcagcattcccttgacactgcccttcgcagagcccgcagcgccccggcagcggcgatagctgcacgcgtggcggggcagacccgcaacattactgtggaccccaggctgtttaaaaagcggcgactccgttcaccccgtgtgctgtttagcacccagcctccccgtgaagctgcagacactcaggatctggacttcgaggtcggtggtgctgcccccttcaacaggactcacaggagcaagcggtcatcatcccatcccatcttccacaggggcgaattctcggtgtgtgacagtgtcagcgtgtgggttggggataagaccaccgccacagacatcaagggcaaggaggtgatggtgttgggagaggtgagcattaacaacagtgtattcaaacagtacttttttgagaccaagtgccgggacccaaatcccgttgacagcgggtgccggggcattgactcaaagcactggaactcatattgtaccacgactcacacctttgtcaaggcgctgaccatggatggcaagcaggctgcctggcggtttatccggatagatacggcctgtatgtgtgtgctcagcaggaaggctgtgagaagagcctgacctgccgacacgctccctccccctgccccttctacactctcctgggcc

SEQ ID NO: 18 - protein, 115 aa, Artificial Sequence
  synthetic
SSSHPIFHRGEFSVVSVWVGDKTTATDIKGKEVMVLGEVNINNSVFKQYFFETKCRDPNPVDSGCRGIDSKHWNSYCTTTHTFALTMDGKQAAWRFIRIDTACVCVLSRKAVRRA